European Patent Specification EP 3 891 306 B1, published February 26, 2025. Title: Biomarker. Applicant: Erber Aktiengesellschaft. The sequence listing filed with the application follows.

SEQUENCE LISTING (50 sequences)

SEQ ID NO: 1 - RNA, 21 nt, Sus scrofa
  microRNA
uggaauguaaagaaguaugua

SEQ ID NO: 2 - RNA, 23 nt, Sus scrofa
  microRNA
ucccugagacccuuuaaccugug

SEQ ID NO: 3 - RNA, 22 nt, Sus scrofa
  microRNA
ucccugagacccuaacuuguga

SEQ ID NO: 4 - RNA, 22 nt, Sus scrofa
  microRNA
ucggauccgucugagcuuggcu

SEQ ID NO: 5 - RNA, 22 nt, Sus scrofa
  microRNA
aagcccuuaccccaaaaagcau

SEQ ID NO: 6 - RNA, 22 nt, Sus scrofa
  microRNA
agcugguaaaauggaaccaaau

SEQ ID NO: 7 - RNA, 23 nt, Sus scrofa
  microRNA
uauggcuuuuuauuccuauguga

SEQ ID NO: 8 - RNA, 23 nt, Sus scrofa
  microRNA
acuccauuuguuuugaugaugga

SEQ ID NO: 9 - RNA, 23 nt, Sus scrofa
  microRNA
uaccacaggguagaaccacggac

SEQ ID NO: 10 - RNA, 22 nt, Sus scrofa
  microRNA
uguaguguuuccuacuuuaugg

SEQ ID NO: 11 - RNA, 21 nt, Sus scrofa
  microRNA
ggugcagugcugcaucucugg

SEQ ID NO: 12 - RNA, 21 nt, Sus scrofa
  microRNA
ugagaacugaauuccauaggc

SEQ ID NO: 13 - RNA, 22 nt, Sus scrofa
  microRNA
aacauucaaccugucggugagu

SEQ ID NO: 14 - RNA, 24 nt, Sus scrofa
  microRNA
uuuggcaaugguagaacucacacu

SEQ ID NO: 15 - RNA, 23 nt, Sus scrofa
  microRNA
uauggcacugguagaauucacug

SEQ ID NO: 16 - RNA, 22 nt, Sus scrofa
  microRNA
ucgugucuuguguugcagccgg

SEQ ID NO: 17 - RNA, 21 nt, Sus scrofa
  microRNA
uagcagcacagaaauauuggc

SEQ ID NO: 18 - RNA, 22 nt, Sus scrofa
  microRNA
uucccuuugucauccuaugccu

SEQ ID NO: 19 - RNA, 22 nt, Sus scrofa
  microRNA
uggaauguaaggaaguguguga

SEQ ID NO: 20 - RNA, 22 nt, Sus scrofa
  microRNA
aagcugccaguugaagaacugu

SEQ ID NO: 21 - RNA, 22 nt, Sus scrofa
  microRNA
aguucuucaguggcaagcuuua

SEQ ID NO: 22 - RNA, 22 nt, Sus scrofa
  microRNA
ucaagagcaauaacgaaaaaug

SEQ ID NO: 23 - RNA, 22 nt, Sus scrofa
  microRNA
uggcagugucuuagcugguugu

SEQ ID NO: 24 - RNA, 21 nt, Sus scrofa
aauaauacaugguugaucuuu

SEQ ID NO: 25 - RNA, 22 nt, Sus scrofa
  microRNA
acuggacuuggagucagaaggc

SEQ ID NO: 26 - RNA, 22 nt, Sus scrofa
  microRNA
cagcagcaauucauguuuugaa

SEQ ID NO: 27 - RNA, 21 nt, Sus scrofa
  microRNA
ucuuggaguaggucauugggu

SEQ ID NO: 28 - RNA, 22 nt, Sus scrofa
  microRNA
uuuugcgauguguuccuaauau

SEQ ID NO: 29 - RNA, 22 nt, Sus scrofa
  microRNA
uuuugcaauauguuccugaaua

SEQ ID NO: 30 - RNA, 22 nt, Sus scrofa
  microRNA
uuuugcgauguguuccuaauac

SEQ ID NO: 31 - RNA, 21 nt, Sus scrofa
  microRNA
gcaguccaugggcauauacac

SEQ ID NO: 32 - RNA, 22 nt, Sus scrofa
  microRNA
uaugugccuuuggacuacaucg

SEQ ID NO: 33 - RNA, 22 nt, Sus scrofa
  microRNA
uccuguacugagcugccccgag

SEQ ID NO: 34 - RNA, 22 nt, Sus scrofa
  microRNA
ugaaggucuacugugugccagg

SEQ ID NO: 35 - RNA, 22 nt, Sus scrofa
  microRNA
uuguacaugguaggcuuucauu

SEQ ID NO: 36 - RNA, 21 nt, Sus scrofa
  microRNA
cagcagcacacugugguuugu

SEQ ID NO: 37 - RNA, 23 nt, Sus scrofa
  microRNA
uagcagcgggaacaguacugcag

SEQ ID NO: 38 - RNA, 22 nt, Sus scrofa
  microRNA
ugugacagauugauaacugaaa

SEQ ID NO: 39 - RNA, 23 nt, Sus scrofa
  microRNA
caacuagacugugagcuucuaga

SEQ ID NO: 40 - RNA, 21 nt, Sus scrofa
  microRNA
uuugugaccugguccacuaac

SEQ ID NO: 41 - RNA, 22 nt, Sus scrofa
  microRNA
aucugucugugucucugagcag

SEQ ID NO: 42 - RNA, 23 nt, Sus scrofa
  microRNA
uauggcuuuucauuccuauguga

SEQ ID NO: 43 - RNA, 22 nt, Sus scrofa
  microRNA
gcucugacuuuauugcacuacu

SEQ ID NO: 44 - RNA, 24 nt, Sus scrofa
  microRNA
uugcaggaacuugugagucuccua

SEQ ID NO: 45 - protein, 309 aa, Artificial Sequence
  Alpha/beta hydrolase domain
MVTSPALRDVHVPHAYPEQQVDLGEITMNYAEAGDPDRPAVLLIPEQTGSWWSYEEAMGLLSEHFHVYAVDLRGQGRSSWTPKRYSLDNFGNDLVRFIALVVKRPVVVAGNSSGGVLAAWLSAYSMPGQLRGVLCEDPPFFASELVPAHGHSVRQGAGPVFELFRTYLGDQWSVGDWEGFCRAAGASASPMARSFVADGIPQHLQEYDPEWARVFYEGTVGLSCPHERMLGQVKTPVLLTHHMRGIDPETGNLLGALSDEQALRARRLMDSAGVTVDYESVPDASHMMHQSAPARYVEIFTRWAAALAP

SEQ ID NO: 46 - protein, 308 aa, Artificial Sequence
  Alpha/beta hydrolase domain
MADPAQRDVYVPHAYPEKQADLGEITMNYAEAGEPDMPAVLLIPEQTGSWWGYEEAMGLLAENFHVYAVDLRGQGRSSWAPKRYSLDNFGNDLVRFIALVVKRPVIVAGNSSGGVLAAWLSAYSMPGQVRGALCEDAPFFASELVTTCGHSIRQAAGPMFELFRTYLGDQWSVGDWTGYCRAADASSSPMARYFVADEIPQHMREYDPEWARAFWEGTVALHCPHEQLLTQVKTPVLLTHHMRDIDPDTGHLVGALSDEQAARARLLMESAGVKVDYASVPDALHMMHQFDPPRYVEIFTQWAATLAA

SEQ ID NO: 47 - protein, 309 aa, Artificial Sequence
  Alpha/beta hydrolase domain
MVTSPALRDVHVPHAYPEQQVDLGEITMNYAEAGDPGRPAVLLIPEQTGSWWSYEEAMGLLAEHFHVYAVDLRGQGRSSWTPKRYSLDNFGNDLVRFIALVVRRPVVVAGNSSGGVLAAWLSAYSMPGQIRGVLCEDPPFFASELVPAHGHSVRQGAGPVFELFRTYLGDQWSVGDWEGFRSAADASASPMARSFVADTIPQHLKEYDPEWARAFYEGTVGLNCPHERMLNRVNTPVLLTHHMRGTDPETGNLLGALSDEQAAQVRRLMESAGVKVDYESVPDASHMMHQSDPARYAEILTPWTAALAP

SEQ ID NO: 48 - protein, 309 aa, Artificial Sequence
  Alpha/beta hydrolase domain
MVTSPALRDVHVPHAYPEQQVDLGEITMNYAEAGDPDRPAVLLIPEQTGSWWSYEEAMGLLAEHFHVYAVDLRGQGRSSWTPKRYSLDNFGNDLVRFIALVVKRPVVVAGNSSGGVLAAWLSAYSMPGQLRGVLCEDPPFFASELVPAHGHSVRQGAGPVFELFRTYLGDQWSVSDWEGFCRAAGASASPMARSFVADGIPQHLKEYDPEWARAFHEGTVGLNCPHERMLGRVNTPVLLTHHMRGTDPETGNLLGALSDEQAAQARLLMESAGVRVDYESVPDASHMMHQSDPARYAEIFTRWAAALAP

SEQ ID NO: 49 - protein, 309 aa, Artificial Sequence
  Alpha/beta hydrolase domain
MVTSPALRDVHVPHAYPEQQVDLGEITMNYAEAGDPGRPAVLLIPEQTGSWWSYEEAMGLLAEHFHVYAVDLRGQGRSSWTPKRYSLDNFGNDLVRFMALVVRRPVVVAGNSSGGVLAAWLSAYSMPGQIRGVLCEDPPFFASELVPAHGHSVRQGAGPVFELFRTYLGDQWSVGDWEGFRSAAGASASPMARSFVADTIPQHLKEYDPEWARAFYEGTVGLNCPHERMLNRVNTPVLLTHHMRGTDPETGNLLGALSDEQAAQARRLMESAGVKVDYESVPDASHMMHQSDPARYAEILTPWAAALAP

SEQ ID NO: 50 - protein, 328 aa, Artificial Sequence
  Alpha/beta hydrolase domain
MAEEGTRSEAADAATQARQLPDSRNIFVSHRFPERQVDLGEVVMNFAEAGSPDNPALLLLPEQTGSWWSYEPVMGLLAENFHVFAVDIRGQGRSTWTPRRYSLDNFGNDLVRFIALVIKRPVVVAGNSSGGLLAAWLSAYAMPGQIRAALCEDAPFFASELVPAYGHSVLQAAGPAFELYRDFLGDQWSIGDWKGFVEAAKASPAKAMQLFPTPDEAPQNLKEYDPEWGRAFFEGTVALHCPHDRMLSQVKTPILITHHARTIDPETGELLGALSDLQAEHAQDIIRSAGVRVDYQSHPDALHMMHLFDPARYAEILTSWSATLPAND